European Patent Application EP 4 215 603 A1, published July 26, 2023. Title: METHODS FOR PRODUCING AUTOLOGOUS T CELLS USEFUL TO TREAT B CELL MALIGNANCIES AND OTHER CANCERS AND COMPOSITIONS THEREOF. Applicant: Kite Pharma, Inc. Application EP. The sequence listing filed with the application follows.

SEQUENCE LISTING (4 sequences)

SEQ ID NO: 1-3 - skipped (3 entries)

SEQ ID NO: 4 - DNA, 5542 bp, synthetic construct
  misc_feature 1..5542: note = Synthetic nucleic acid sequence of MSGV1 gamma retroviral vector backbone
  source 1..5542: mol_type = other DNA
ggatccgataaaataaaagattttatttagtctccagaaaaaggggggaatgaaagaccccacctgtaggtttggcaagctagcttaagtaacgccattttgcaaggcatggaaaatacataactgagaatagagaagttcagatcaaggttaggaacagagagacagcagaatatgggccaaacaggatatctgtggtaagcagttcctgccccggctcagggccaagaacagatggtccccagatgcggtcccgccctcagcagtttctagagaaccatcagatgtttccagggtgccccaaggacctgaaaatgaccctgtgccttatttgaactaaccaatcagttcgcttctcgcttctgttcgcgcgcttctgctccccgagctcaataaaagagcccacaacccctcactcggcgcgccagtcctccgatagactgcgtcgcccgggtacccgtgtatccaataaaccctcttgcagttgcatccgacttgtggtctcgctgttccttgggagggtctcctctgagtgattgactacccgtcagcgggggtctttcatgggtaacagtttcttgaagttggagaacaacattctgagggtaggagtcgaatattaagtaatcctgactcaattagccactgttttgaatccacatactccaatactcctgaaatccatcgatggagttcattatggacagcgcagaaagagctggggagaattgtgaaattgttatccgctcacaattccacacaacatacgagccggaagcataaagtgtaaagcctggggtgcctaatgagtgagctaactcacattaattgcgttgcgctcactgcccgctttccagtcgggaaacctgtcgtgccagctgcattaatgaatcggccaacgcgcggggagaggcggtttgcgtattgggcgctcttccgcttcctcgctcactgactcgctgcgctcggtcgttcggctgcggcgagcggtatcagctcactcaaaggcggtaatacggttatccacagaatcaggggataacgcaggaaagaacatgtgagcaaaaggccagcaaaaggccaggaaccgtaaaaaggccgcgttgctggcgtttttccataggctccgcccccctgacgagcatcacaaaaatcgacgctcaagtcagaggtggcgaaacccgacaggactataaagataccaggcgtttccccctggaagctccctcgtgcgctctcctgttccgaccctgccgcttaccggatacctgtccgcctttctcccttcgggaagcgtggcgctttctcatagctcacgctgtaggtatctcagttcggtgtaggtcgttcgctccaagctgggctgtgtgcacgaaccccccgttcagcccgaccgctgcgccttatccggtaactatcgtcttgagtccaacccggtaagacacgacttatcgccactggcagcagccactggtaacaggattagcagagcgaggtatgtaggcggtgctacagagttcttgaagtggtggcctaactacggctacactagaaggacagtatttggtatctgcgctctgctgaagccagttaccttcggaaaaagagttggtagctcttgatccggcaaacaaaccaccgctggtagcggtggtttttttgtttgcaagcagcagattacgcgcagaaaaaaaggatctcaagaagatcctttgatcttttctacggggtctgacgctcagtggaacgaaaactcacgttaagggattttggtcatgagattatcaaaaaggatcttcacctagatccttttaaattaaaaatgaagttttaaatcaatctaaagtatatatgagtaaacttggtctgacagttaccaatgcttaatcagtgaggcacctatctcagcgatctgtctatttcgttcatccatagttgcctgactccccgtcgtgtagataactacgatacgggagggcttaccatctggccccagtgctgcaatgataccgcgagacccacgctcaccggctccagatttatcagcaataaaccagccagccggaagggccgagcgcagaagtggtcctgcaactttatccgcctccatccagtctattaattgttgccgggaagctagagtaagtagttcgccagttaatagtttgcgcaacgttgttgccattgctacaggcatcgtggtgtcacgctcgtcgtttggtatggcttcattcagctccggttcccaacgatcaaggcgagttacatgatcccccatgttgtgcaaaaaagcggttagctccttcggtcctccgatcgttgtcagaagtaagttggccgcagtgttatcactcatggttatggcagcactgcataattctcttactgtcatgccatccgtaagatgcttttctgtgactggtgagtactcaaccaagtcattctgagaatagtgtatgcggcgaccgagttgctcttgcccggcgtcaatacgggataataccgcgccacatagcagaactttaaaagtgctcatcattggaaaacgttcttcggggcgaaaactctcaaggatcttaccgctgttgagatccagttcgatgtaacccactcgtgcacccaactgatcttcagcatcttttactttcaccagcgtttctgggtgagcaaaaacaggaaggcaaaatgccgcaaaaaagggaataagggcgacacggaaatgttgaatactcatactcttcctttttcaatattattgaagcatttatcagggttattgtctcatgagcggatacatatttgaatgtatttagaaaaataaacaaataggggttccgcgcacatttccccgaaaagtgccacctgacgtctaagaaaccattattatcatgacattaacctataaaaataggcgtatcacgaggccctttcgtctcgcgcgtttcggtgatgacggtgaaaacctctgacacatgcagctcccggagacggtcacagcttgtctgtaagcggatgccgggagcagacaagcccgtcagggcgcgtcagcgggtgttggcgggtgtcggggctggcttaactatgcggcatcagagcagattgtactgagagtgcaccatatgcggtgtgaaataccgcacagatgcgtaaggagaaaataccgcatcaggcgccattcgccattcaggctgcgcaactgttgggaagggcgatcggtgcgggcctcttcgctattacgccagctggcgaaagggggatgtgctgcaaggcgattaagttgggtaacgccagggttttcccagtcacgacgttgtaaaacgacggccagtgccacgctctcccttatgcgactcctgcattaggaagcagcccagtagtaggttgaggccgttgagcaccgccgccgcaaggaatggtgcatgcaaggagatggcgcccaacagtcccccggccacggggcctgccaccatacccacgccgaaacaagcgctcatgagcccgaagtggcgagcccgatcttccccatcggtgatgtcggcgatataggcgccagcaaccgcacctgtggcgccggtgatgccggccacgatgcgtccggcgtagaggcgatttaaagacaggatatcagtggtccaggctctagttttgactcaacaatatcaccagctgaagcctatagagtacgagccatagataaaataaaagattttatttagtctccagaaaaaggggggaatgaaagaccccacctgtaggtttggcaagctagcttaagtaacgccattttgcaaggcatggaaaatacataactgagaatagagaagttcagatcaaggttaggaacagagagacagcagaatatgggccaaacaggatatctgtggtaagcagttcctgccccggctcagggccaagaacagatggtccccagatgcggtcccgccctcagcagtttctagagaaccatcagatgtttccagggtgccccaaggacctgaaaatgaccctgtgccttatttgaactaaccaatcagttcgcttctcgcttctgttcgcgcgcttctgctccccgagctcaataaaagagcccacaacccctcactcggcgcgccagtcctccgatagactgcgtcgcccgggtacccgtattcccaataaagcctcttgctgtttgcatccgaatcgtggactcgctgatccttgggagggtctcctcagattgattgactgcccacctcgggggtctttcatttggaggttccaccgagatttggagacccctgcctagggaccaccgacccccccgccgggaggtaagctggccagcggtcgtttcgtgtctgtctctgtctttgtgcgtgtttgtgccggcatctaatgtttgcgcctgcgtctgtactagttagctaactagctctgtatctggcggacccgtggtggaactgacgagttcggaacacccggccgcaaccctgggagacgtcccagggacttcgggggccgtttttgtggcccgacctgagtccaaaaatcccgatcgttttggactctttggtgcaccccccttagaggagggatatgtggttctggtaggagacgagaacctaaaacagttcccgcctccgtctgaatttttgctttcggtttgggaccgaagccgcgccgcgcgtcttgtctgctgcagcatcgttctgtgttgtctctgtctgactgtgtttctgtatttgtctgagaatatgggcccgggctagcctgttaccactcccttaagtttgaccttaggtcactggaaagatgtcgagcggatcgctcacaaccagtcggtagatgtcaagaagagacgttgggttaccttctgctctgcagaatggccaacctttaacgtcggatggccgcgagacggcacctttaaccgagacctcatcacccaggttaagatcaaggtcttttcacctggcccgcatggacacccagaccaggtcccctacatcgtgacctgggaagccttggcttttgacccccctccctgggtcaagccctttgtacaccctaagcctccgcctcctcttcctccatccgccccgtctctcccccttgaacctcctcgttcgaccccgcctcgatcctccctttatccagccctcactccttctctaggcgcccccatatggccatatgagatcttatatggggcacccccgccccttgtaaacttccctgaccctgacatgacaagagttactaacagcccctctctccaagctcacttacaggctctctacttagtccagcacgaagtctggagacctctggcggcagcctaccaagaacaactggaccgaccggtggtacctcacccttaccgagtcggcgacacagtgtgggtccgccgacaccagactaagaacctagaacctcgctggaaaggaccttacacagtcctgctgaccacccccaccgccctcaaagtagacggcatcgcagcttggatacacgccgcccacgtgaaggctgccgaccccgggggtggaccatcctctag